European Patent Application EP 4 541 808 A1, published April 23, 2025. Title: L-Histidine Export Protein and Method of Producing L-Histidine Using the Same. Applicant: CJ CheilJedang Corporation. The sequence listing filed with the application follows.

SEQUENCE LISTING (48 sequences)

SEQ ID NO: 1 - protein, 314 aa, synthetic construct
  REGION 1..314: note = synthetic_Haq protein
MKSKNATLVGLSAVVLWSAIVGLIRGVSEHLGATGGAAAIYTVASLILLVSVGFPRLASFPRRYLLWGSVLFVAYELCLSLSIGYAHTGRQAIEVGMVNYLWPTFTLVAAILFGGQRATLLVVPGFILSMLGICWVLGGDQGLDPSGMLANIRDNPLSYGLAFIGALIWAAYCTVTTRIAQGQNGVTPFFMLVALALWVKVLLGGHVAELSFSVPALVYLVLAAAAMGLGYAAWNVGILHGNVTVLAGASYFIPVFSSALSALLLRAPLPTSFWVGAALVCAGSILCWRATRSLDLSKEPAARAARPEGPPQNQ

SEQ ID NO: 2 - DNA, 945 bp, synthetic construct
  misc_feature 1..945: note = synthetic_Haq gene encoding Haq protein
  source 1..945: mol_type = other DNA
atgaagagcaagaacgcaaccctggtcggattgagcgcggtggtactgtggagtgccatcgtgggcctgatccgtggcgtgagcgagcatctcggagccaccggcggggcggcggccatttacacggtggcttcgctgatcctgctggtgtcggtgggattcccgcgcctggcgagtttcccgcgcaggtatctgctatggggcagcgtgctgttcgtggcttatgaattgtgcctgtcgctctcgatcggttatgcccataccggccgccaggccatcgaagtcggcatggtcaattacctctggccgaccttcaccctggtggcggccatcctcttcggaggccagcgcgccacgctgctggtggtgccaggcttcatcctttccatgctgggcatctgctgggtgctcgggggcgaccaggggctggatccttccggcatgctggccaatatccgtgacaatccgctgagctacggcctggccttcatcggggccttgatctgggcggcctactgcaccgtgactacccgcatcgcccaaggccagaacggggtgacgcctttcttcatgctggtggcattggcattgtgggtgaaggtgctgctgggcgggcatgtggctgaactatccttcagtgtgcccgcactggtctacctggtgctggctgcggcggcgatggggctgggctatgcggcctggaacgtgggcatcctgcatggcaatgtgacagtgctggccggtgcctcgtatttcatcccggtcttttcttcggccttgtcggccttgctgctacgtgcgccgctgcccacctcgttctgggtgggcgctgcgctggtgtgcgccgggtcgatcctgtgctggcgggctacccgcagcctggatttgtcaaaagaacctgcagcgcgggcggcacgtcccgaaggcccacctcagaaccaatag

SEQ ID NO: 3 - protein, 312 aa, synthetic construct
  REGION 1..312: note = synthetic_Cpi protein
MQSTRKATLIGLIAILLWSSIVGLIRGVSESLGATGGAAMMYSVASVLLMLTVGFVRLREFPRRYLVWGSILFVSYELCLSLSIGYSHSGRQAIEVGMVNYLWPSFTMLCAIAFNKQKANVLIVPGFLIAILGICLVLGGEQGLDVAGMVANVRDNPLSYGLALAGALIWAAYCTVTNRIAGGNNGVTLFFMLTAMALWIKYFTGDHAPMAFTYHAVIYLALAASAMGFGYPAWNVGILHGNVTVLAGASYFIPVISAALAGLLLHIPLSLAFWKGASLVCAGSVLCWLATRARKVAATPDRAPVRDRVWKQ

SEQ ID NO: 4 - DNA, 939 bp, synthetic construct
  misc_feature 1..939: note = synthetic_Cpi gene encoding Cpi protein
  source 1..939: mol_type = other DNA
atgcaaagcacgcgtaaggccacgttgatcgggctcattgcgatcctgttgtggagttccatcgtcggcctgatccgcggcgtcagtgaaagcctcggcgcgaccggtggcgccgccatgatgtactcggttgcctccgtcctgcttatgctgacggttggcttcgtgcgtctgcgcgaatttccgcggcgctatctggtctggggcagcatcctgttcgtctcctacgaactgtgcctgtcgctgtccatcggctattcgcacagcggcaggcaggcgatcgaggtggggatggtcaattacctctggccgtctttcaccatgttgtgcgccatcgccttcaacaagcagaaggcgaacgttctgatcgtgccgggcttcctgattgcgatcctgggtatctgcctggtgctgggcggcgagcagggtctggatgttgcaggcatggtggccaatgtcagggacaatccgctcagctacggcctcgctttagcgggcgcgctgatctgggcggcctattgcaccgtgaccaacaggattgccggcggcaacaacggcgtcacgctgtttttcatgctcaccgcaatggcgctgtggatcaagtacttcaccggcgaccatgcgccgatggctttcacataccacgccgtcatctacctggcactggcagcgtcggcgatgggcttcggctacccggcgtggaacgtgggcatcctgcacggcaacgtaacggtgcttgccggcgcgtcgtatttcatccctgtgatttcagccgcactggctggcttgctcttgcatataccgctttcgctggcgttctggaaaggcgcgtcgctggtatgcgcggggtccgtgctgtgctggttggcgacgcgcgcgcgcaaggtggctgcaacgcccgaccgtgctccggtccgcgaccgtgtctggaagcaatga

SEQ ID NO: 5 - protein, 293 aa, synthetic construct
  REGION 1..293: note = synthetic_Kcr protein
MDKKRATLIGFSAIILWSTMVGLIRGVSEGLGPVGGAAMIYSLSGLLLIFTVGFPQLRQIPPRYLLVGSLFFVSYEMCLALSLGYAGTRQQAIEVGMVNYLWPSLTILFAIIFNGQKTTWLVIPGLLLSIVGVTWVLGGEHGLDLAEIRSNVISSPLSYILAFVGAFIWAAYCTVTAKYAKGKNGITLFVLFTALALWVKFLMSEQPPMIFSWPVVIKLVTCALALGFAYAAWNVGILHGNVSLLAAASYFTPVLSSALAAFLLSAALSWSFWQGAAMVCGGSLLCWYATRRP

SEQ ID NO: 6 - DNA, 371 bp, synthetic construct
  misc_feature 1..371: note = synthetic_Kcr gene encoding Kcr protein
  source 1..371: mol_type = other DNA
atggataagaaaagagcgacgctcattggatttagcgccattattttgtggagtacgatggtgggtctgattcgcggcgtaagcgaagggctcggcccggtgggcggagccgcaatgatttacagcctcagcggcctgctgctgatttttaccgttggcttcccacaattgcgccaaattccaccgcgctatttgctggtaggtagcctgttttttgtcagctacgaaatgtgcctcgcgctctcattaggctatgccggcactcgccaacaggccatcgaagtcggcatggtgaattatctctggcctagcctgacgattttatttgcgattatctttaatggtcaaaaaaccacctggctggttatccc

SEQ ID NO: 7 - protein, 238 aa, synthetic construct
  REGION 1..238: note = synthetic_Cst protein
MSTLSILIAGFALGLSLIVAIGPQNALLIKQGIKREHVWVVIAICAVSDIILISGGTAGVGYLVETFPTALVVLKYLGAIYLAYFTYLCFRDALRDKVETLSPAQIEPNKTQQIDAFDGGDLGGSSVDTRRRTTRLRQQVRQSTWVKPALATLAICWLNPAAYVDVLVMIGGLANQYGETGRWFFAAGAIAASMLWFPSVGLAAAKFSHVLSRPAVWRGINFGIGCIMALLTIKLLLT

SEQ ID NO: 8 - DNA, 717 bp, synthetic construct
  misc_feature 1..717: note = synthetic_Cst gene encoding Cst protein
  source 1..717: mol_type = other DNA
atgtcaacgctgtctatcctcatcgccggtttcgcactagggctctcacttatcgtagcgattggcccgcaaaatgctctgctgatcaaacagggcattaaacgcgagcacgtgtgggtagtcattgcgatttgcgcggtgtccgacattattttgattagcggtggcaccgcgggggtgggctatctggtggagactttcccgaccgcactggtggtgctgaagtatctgggcgcgatttatctggcttactttacttatctgtgctttcgcgatgcgttgcgcgacaaggttgaaactctctcccctgcgcagatcgagccgaataagacgcagcagatcgatgcattcgatggcggcgacttgggcggttcttctgttgatacccggcggcgcaccacgcgtctgcgccagcaagtacgccaatcgacctgggtgaagccagctcttgcgaccttggcgatttgctggctgaacccggcagcttatgtcgatgtgctggtaatgattggcggacttgccaaccaatacggcgaaaccggccgatggttttttgctgccggtgccattgcagcgagcatgctgtggtttcccagcgttggtcttgctgccgcgaagttctcgcacgtactttcgcgccctgcggtatggcgcggcatcaacttcggcattggctgcatcatggcgctgctgaccattaagctgctgttgacctag

SEQ ID NO: 9 - protein, 242 aa, synthetic construct
  REGION 1..242: note = synthetic_LsaF protein
MSPSHDPLPRRAGAAAGLRDSLGVGLGIFPLGIALGILVIQAGLPWWLAPALSIGIFAGSVELLLVSMLAAATPLVTIAATVFAVNFRHVFYAFSFPLSRVRPGLPRAYSIYAMIDEAYATYVLMDPDRLSSARMVTGQLAMQLYWVLGGFVGIMIANVLPAPIEGFEFALVALFVVMSMDAIRGKRELPSALLACLAVTVAILVAGDNALLVALALYSGLLGLRYFLTKRTTDTAEEGERA

SEQ ID NO: 10 - protein, 140 aa, synthetic construct
  REGION 1..140: note = synthetic_LsaE protein
MRCWSRLRCTPGYWGCAISSPSEPRTLRRRASVPSTEYLIAGVVVAGLITLALRALPFAALKPLRKSKLVQALGRWMPAGILVILAVVVLRDQLISQQGRVWPVLVATAITALAHLLSKRRALVSIAAGTACYVLLLNFF

SEQ ID NO: 11 - DNA, 1048 bp, synthetic construct
  misc_feature 1..1048: note = synthetic_Isa gene
  source 1..1048: mol_type = other DNA
atgtctccgtcacacgatcctttaccgcgccgcgcgggcgccgcggccggccttcgagattctctcggggtcggcctcggcattttccccttgggcattgccctcggaattcttgtcattcaggcgggacttccctggtggctcgccccggccctctcgattggtatcttcgcgggatctgtcgagctgctcctggtcagcatgctcgccgccgcgactccgctcgtgacgatcgccgcgaccgtgttcgccgtgaactttcggcacgtattctacgcgttctcgtttccgctttcgcgggtgcgaccgggtctaccccgggcgtactccatctacgcaatgatcgacgaggcctacgccacctatgtgctgatggatccggatcgcctgagctcagcccgcatggtaaccggccagctcgcgatgcagctctattgggtgctcggcggcttcgtcggcatcatgattgcgaacgtgctccctgcccccattgagggctttgagtttgcactcgtggcgctcttcgtggtgatgtcgatggatgcgattcgcggcaagcgcgagctcccatcggccttgctggcttgcctcgctgtcacggttgcaatactggtcgctggcgacaatgcgctgctggtcgcgcttgcgctgtactccgggctactggggctgcgctatttcctcaccaagcgaaccacggacactgcggaggagggcgagcgtgcctagcaccgaatatctaatcgcgggcgtcgtcgtcgcgggcctcatcaccctggcgctgcgcgcactcccgtttgcggcgctcaaaccgctgcgcaaatctaagctcgtgcaggcgctcgggcgctggatgcccgctggcatcctcgttatcctcgccgtcgtcgtactgcgcgatcagctcatatcgcagcagggccgggtgtggccggtgctcgtcgcgaccgcgatcacggccctcgctcacttgctctcaaagcgacgcgcgctcgtgagcatcgcggctggcaccgcctgctacgtgctgctgctcaactttttctag

SEQ ID NO: 12 - protein, 251 aa, synthetic construct
  REGION 1..251: note = synthetic_DvaF protein
MSVEAQPGANDRPYSVRHEITQGALLILPAGLGMIPIGIAFGLLVVQSGLPWWMAPALSFFAYAGSLELLLITLITSLTPLVTIAAASFFVNFRHVFYAFNFPLKVVTNPFLKFYAMYSLTDEIFAVTVANPKGWTQPRVISAGAVLQICWVGGGLMGVLLSSFIPFQIRGLSFALCALFITLTLDACRTKQEIPSLLLGAAAFGFALLLLPSQPIFAAMIGFVATLAARYTIAVRLTRPLPAEMESDDAA

SEQ ID NO: 13 - protein, 111 aa, synthetic construct
  REGION 1..111: note = synthetic_DvaE protein
MQLDIPFWYLASVLLIAFAVTFTLRALPFAILEPLRKSQFVRVMAVWMPAGILVILALATFKSTLAEEPGGLVHLLIASGVTIAVHLFGGRRTLVSVAAGTLAFVLLVNFF

SEQ ID NO: 14 - DNA, 756 bp, synthetic construct
  misc_feature 1..756: note = synthetic_DvaF gene encoding DvaF protein
  source 1..756: mol_type = other DNA
atgagcgttgaggcgcagcctggcgcaaacgaccgaccctatagcgtgcgccacgagatcacgcagggcgcactcctgattctccccgcagggctcggaatgattccgatcggcattgccttcggcctgcttgtggtgcaatcggggctcccgtggtggatggcacccgccctttcgttcttcgcgtacgcgggctcactcgagcttctgctcatcacgctcatcacgtcgcttacgccgcttgtaacgatcgctgcggcatcgttcttcgtgaacttccgccacgtgttctacgcgtttaatttcccgctcaaggtcgtcacgaacccgttcttgaagttctacgcgatgtactccctcaccgacgagatcttcgcggtaacggttgccaatccaaaggggtggacgcagccgcgcgtgatctcggcaggggccgtactccagatctgctgggtgggtggcggcctcatgggggtactgctctcgagcttcatccccttccagatccgcggcctgagtttcgcgctgtgcgccctgttcatcacgctgaccctcgatgcgtgccgcacgaaacaggagatcccgtcacttctcctcggtgctgccgccttcggtttcgcgctccttttgctcccgagccagccgatcttcgccgcgatgattggcttcgtggcgaccctcgccgcgcgctacacgatcgccgtgcgcctcacgaggccactcccggcagagatggagagcgacgatgcagcttga

SEQ ID NO: 15 - DNA, 335 bp, synthetic construct
  misc_feature 1..335: note = synthetic_DvaE gene encoding DvaE protein
  source 1..335: mol_type = other DNA
atgcagcttgacatccccttctggtatctcgcctcggttctcctcatcgccttcgccgtgaccttcacgctgcgcgcgctcccgttcgcgattctcgaaccactgcgcaaatcgcaattcgtgcgcgtcatggccgtgtggatgcccgcgggcatcctcgtgatcctcgcgctcgcgacctttaagagcaccctcgccgaggaacccggtggtctcgttcacctgctgatcgcctcaggagtcacgattgccgtgcacctcttcggtggtcgccgcaccctcgtgagcgtcgccgcgggcaccctcgccttcgtgctgctcgtgaactttttcta

SEQ ID NO: 16 - DNA, 1081 bp, synthetic construct
  misc_feature 1..1081: note = synthetic_DvaFE gene
  source 1..1081: mol_type = other DNA
atgagcgttgaggcgcagcctggcgcaaacgaccgaccctatagcgtgcgccacgagatcacgcagggcgcactcctgattctccccgcagggctcggaatgattccgatcggcattgccttcggcctgcttgtggtgcaatcggggctcccgtggtggatggcacccgccctttcgttcttcgcgtacgcgggctcactcgagcttctgctcatcacgctcatcacgtcgcttacgccgcttgtaacgatcgctgcggcatcgttcttcgtgaacttccgccacgtgttctacgcgtttaatttcccgctcaaggtcgtcacgaacccgttcttgaagttctacgcgatgtactccctcaccgacgagatcttcgcggtaacggttgccaatccaaaggggtggacgcagccgcgcgtgatctcggcaggggccgtactccagatctgctgggtgggtggcggcctcatgggggtactgctctcgagcttcatccccttccagatccgcggcctgagtttcgcgctgtgcgccctgttcatcacgctgaccctcgatgcgtgccgcacgaaacaggagatcccgtcacttctcctcggtgctgccgccttcggtttcgcgctccttttgctcccgagccagccgatcttcgccgcgatgattggcttcgtggcgaccctcgccgcgcgctacacgatcgccgtgcgcctcacgaggccactcccggcagagatggagagcgacgatgcagcttgacatccccttctggtatctcgcctcggttctcctcatcgccttcgccgtgaccttcacgctgcgcgcgctcccgttcgcgattctcgaaccactgcgcaaatcgcaattcgtgcgcgtcatggccgtgtggatgcccgcgggcatcctcgtgatcctcgcgctcgcgacctttaagagcaccctcgccgaggaacccggtggtctcgttcacctgctgatcgcctcaggagtcacgattgccgtgcacctcttcggtggtcgccgcaccctcgtgagcgtcgccgcgggcaccctcgccttcgtgctgctcgtgaactttttctaa

SEQ ID NO: 17 - DNA, 409 bp, synthetic construct
  misc_feature 1..409: note = synthetic_PgapA
  source 1..409: mol_type = other DNA
tctgagactttaatttgtggattcacgggggtgtaatgtagttcataattaaccccattcgggggagcagatcgtagtgcgaacgatttcaggttcgttccctgcaaaaactatttagcgcaagtgttggaaatgcccccgtttggggtcaatgtccatttttgaatgtgtctgtatgattttgcatctgctgcgaaatctttgtttccccgctaaagttgaggacaggttgacacggagttgactcgacgaattatccaatgtgagtaggtttggtgcgtgagttggaaaaattcgccatactcgcccttgggttctgtcagctcaagaattcttgagtgaccgatgctctgattgacctaactgcttgacacattgcatttcctacaatctttagaggagacacaac

SEQ ID NO: 18 - DNA, 40 bp, synthetic construct
  misc_feature 1..40: note = synthetic_primer
  source 1..40: mol_type = other DNA
gtacccggggatcctctagacaaagccgaagagaagttgg

SEQ ID NO: 19 - DNA, 30 bp, synthetic construct
  misc_feature 1..30: note = synthetic_primer
  source 1..30: mol_type = other DNA
gcatagagtactcggcgcccataaatttca

SEQ ID NO: 20 - DNA, 30 bp, synthetic construct
  misc_feature 1..30: note = synthetic_primer
  source 1..30: mol_type = other DNA
gcgccgagtactctatgccgagaagttgaa

SEQ ID NO: 21 - DNA, 40 bp, synthetic construct
  misc_feature 1..40: note = synthetic_primer
  source 1..40: mol_type = other DNA
gcctgcaggtcgactctagactgggcatcacactattttt

SEQ ID NO: 22 - DNA, 531 bp, synthetic construct
  misc_feature 1..531: note = synthetic_del-N2131L
  source 1..531: mol_type = other DNA
gtacccggggatcctctagacaaagccgaagagaagttggcttgacggacccgaaattccagctgattttgacgatcctgatgcacccggcaggtggcctggcgaaaagttggggcttcctcaagaaggggccggctctctgtcctcagtggctcgtcgtatcggcggggtctgcgtggactggggtgtttcctgggttattgctattgtgctgtccaatttcacggatgtgctgggcgatgtagcgacatccacgctcattattttcgtgatcctgggttggcttaccggttggatctttgctcgcaccccaggtcatgccgtgtttggcatgggccttgcgcgtgtggatgcagaggaacgtgtgggctggtggcgtgcgctggttcgcccactgctgacgatcttgattctgcctgccgtgatggtggatgctgacggccgtgggctccacgacaaggcaacgggaactgcagttatccgcgggtaatttgtcttgagtgaaatttatgggcgccgagtactctatgc

SEQ ID NO: 23 - DNA, 555 bp, synthetic construct
  misc_feature 1..555: note = synthetic_del-N2131R
  source 1..555: mol_type = other DNA
gcgccgagtactctatgccgagaagttgaacagcaatcttgcagcaactcctcagtattcacaccagccccaatggacacaaaaacatcagccccagaatcgcccctaagggcctcaaatacacgatctggaccaactagtcatcgggaaaacccaaccccttaaatcgccttctgcgcttaaggggtcaatgctagataagtaggaacaacaacgtttgggcggccaggatctttgcgatcatcgccagcggatacacagaggtataacccatggcagggagctcgttgcgggaggcatctgacacataactcagcacagcagggtgggtttgcgtaccggcgaggatgccagcggtttcaccgaaggggattttcatcagtttgtggccaacgaacagcaccgtgatggagatgaacaaagtgagcagcgcaccgaagccgatgatggtgagtgattgggggtcgctgatcgctgatcgaaatcctgcgcccgctgaggtaccgatggcagccaaaaatagtgtgatgcccagtctagagtcgacctgcaggc

SEQ ID NO: 24 - DNA, 30 bp, synthetic construct
  misc_feature 1..30: note = synthetic_Haq-F
  source 1..30: mol_type = other DNA
aggagacacaacatgaagagcaagaacgca

SEQ ID NO: 25 - DNA, 40 bp, synthetic construct
  misc_feature 1..40: note = synthetic_Haq-R
  source 1..40: mol_type = other DNA
tcaacttctcggcatagagtctattggttctgaggtgggc

SEQ ID NO: 26 - DNA, 40 bp, synthetic construct
  misc_feature 1..40: note = synthetic_PgapA-F
  source 1..40: mol_type = other DNA
gaaatttatgggcgccgagttctgagactttaatttgtgg

SEQ ID NO: 27 - DNA, 30 bp, synthetic construct
  misc_feature 1..30: note = synthetic_PgapA-R
  source 1..30: mol_type = other DNA
cttgctcttcatgttgtgtctcctctaaag

SEQ ID NO: 28 - DNA, 30 bp, synthetic construct
  misc_feature 1..30: note = synthetic_Cpi-F
  source 1..30: mol_type = other DNA
aggagacacaacatgcaaagcacgcgtaag

SEQ ID NO: 29 - DNA, 40 bp, synthetic construct
  misc_feature 1..40: note = synthetic_Cpi-R
  source 1..40: mol_type = other DNA
tcaacttctcggcatagagttcattgcttccagacacggt

SEQ ID NO: 30 - DNA, 30 bp, synthetic construct
  misc_feature 1..30: note = synthetic_PgapA-R
  source 1..30: mol_type = other DNA
cgtgctttgcatgttgtgtctcctctaaag

SEQ ID NO: 31 - DNA, 30 bp, synthetic construct
  misc_feature 1..30: note = synthetic_Kcr-F
  source 1..30: mol_type = other DNA
aggagacacaacatggataagaaaagagcg

SEQ ID NO: 32 - DNA, 40 bp, synthetic construct
  misc_feature 1..40: note = synthetic_Kcr-R
  source 1..40: mol_type = other DNA
tcaacttctcggcatagagtttagggacggcgggtggcgt

SEQ ID NO: 33 - DNA, 30 bp, synthetic construct
  misc_feature 1..30: note = synthetic_PgapA-R
  source 1..30: mol_type = other DNA
tttcttatccatgttgtgtctcctctaaag

SEQ ID NO: 34 - DNA, 30 bp, synthetic construct
  misc_feature 1..30: note = synthetic_Cst-F
  source 1..30: mol_type = other DNA
aggagacacaacatgtcaacgctgtctatc

SEQ ID NO: 35 - DNA, 40 bp, synthetic construct
  misc_feature 1..40: note = synthetic_Cst-R
  source 1..40: mol_type = other DNA
tcaacttctcggcatagagtctaggtcaacagcagcttaa

SEQ ID NO: 36 - DNA, 30 bp, synthetic construct
  misc_feature 1..30: note = synthetic_PgapA-R
  source 1..30: mol_type = other DNA
cagcgttgacatgttgtgtctcctctaaag

SEQ ID NO: 37 - DNA, 30 bp, synthetic construct
  misc_feature 1..30: note = synthetic_Isa-F
  source 1..30: mol_type = other DNA
aggagacacaacatgtctccgtcacacgat

SEQ ID NO: 38 - DNA, 40 bp, synthetic construct
  misc_feature 1..40: note = synthetic_Isa-R
  source 1..40: mol_type = other DNA
tcaacttctcggcatagagtctagaaaaagttgagcagca

SEQ ID NO: 39 - DNA, 30 bp, synthetic construct
  misc_feature 1..30: note = synthetic_PgapA-R
  source 1..30: mol_type = other DNA
tgacggagacatgttgtgtctcctctaaag

SEQ ID NO: 40 - DNA, 30 bp, synthetic construct
  misc_feature 1..30: note = synthetic_Dva-F
  source 1..30: mol_type = other DNA
aggagacacaacatgagcgttgaggcgcag

SEQ ID NO: 41 - DNA, 40 bp, synthetic construct
  misc_feature 1..40: note = synthetic_Dva-R
  source 1..40: mol_type = other DNA
tcaacttctcggcatagagtttagaaaaagttcacgagca

SEQ ID NO: 42 - DNA, 30 bp, synthetic construct
  misc_feature 1..30: note = synthetic_PgapA-R
  source 1..30: mol_type = other DNA
ctcaacgctcatgttgtgtctcctctaaag

SEQ ID NO: 43 - DNA, 100 bp, synthetic construct
  misc_feature 1..100: note = synthetic_PyccA
  source 1..100: mol_type = other DNA
ttccagatcaaatgcgtaaagatgggtaaaacttctgggtgcccttacgcattatcattatgctgcttaattaattacatctgtcatagagagtgactca

SEQ ID NO: 44 - DNA, 38 bp, synthetic construct
  misc_feature 1..38: note = synthetic_Dva-F
  source 1..38: mol_type = other DNA
ctgtcatagagagtgactcaatgagcgttgaggcgcag

SEQ ID NO: 45 - DNA, 40 bp, synthetic construct
  misc_feature 1..40: note = synthetic_Dva-R
  source 1..40: mol_type = other DNA
cgggtaccgagctcgaattcttagaaaaagttcacgagca

SEQ ID NO: 46 - DNA, 40 bp, synthetic construct
  misc_feature 1..40: note = synthetic_PyccA-F
  source 1..40: mol_type = other DNA
actcactatagggcgaattcttccagatcaaatgcgtaaa

SEQ ID NO: 47 - DNA, 30 bp, synthetic construct
  misc_feature 1..30: note = synthetic_PyccA-R
  source 1..30: mol_type = other DNA
tgagtcactctctatgacagatgtaattaa

SEQ ID NO: 48 - protein, 111 aa, synthetic construct
  REGION 1..111: note = synthetic_DvaE protein (R92C var.)
MQLDIPFWYLASVLLIAFAVTFTLRALPFAILEPLRKSQFVRVMAVWMPAGILVILALATFKSTLAEEPGGLVHLLIASGVTIAVHLFGGRCTLVSVAAGTLAFVLLVNFF